European Patent Specification EP 3 576 781 B9, published March 6, 2024. Title: NEOANTIGENS AND USES THEREOF FOR TREATING CANCER. Applicant: Icahn School of Medicine at Mount Sinai The Simons Center for Systems Biology at the Institute for Advanced Study Memorial Sloan Kettering Cancer Center Universitat zu Koln Luksza, Marta Balachandran, Vinod P. Levine, Arnold J. Wolchok, Jedd D. Merghoub, Taha Leach, Steven D. Chan, Timothy A. Greenbaum, Benjamin D. Laessig, Michael. Application Filed herewith. The sequence listing filed with the application follows.

SEQUENCE LISTING (152 sequences)

SEQ ID NO: 1 - protein, 9 aa, Artificial Sequence
  Neoantigenic peptide
VMKHLLSPL

SEQ ID NO: 2 - protein, 9 aa, Artificial Sequence
  Neoantigenic peptide
MHHPGSRKF

SEQ ID NO: 3 - protein, 9 aa, Artificial Sequence
  Neoantigen peptide
NSTLIPTLI

SEQ ID NO: 4 - protein, 9 aa, Artificial Sequence
  Neoantigenic peptide
SSSGVNSTI

SEQ ID NO: 5 - protein, 9 aa, Artificial Sequence
  Neoantigenic peptide
STLIPTLIL

SEQ ID NO: 6 - protein, 9 aa, Artificial Sequence
  Neoantigenic peptide
AEASSAVPT

SEQ ID NO: 7 - protein, 9 aa, Artificial Sequence
  Neoantigenic peptide
EASSAVPTV

SEQ ID NO: 8 - protein, 9 aa, Artificial Sequence
  Neoantigenic peptide
SRAVTSTTI

SEQ ID NO: 9 - protein, 9 aa, Artificial Sequence
  Neoantigenic peptide
STTIPILTL

SEQ ID NO: 10 - protein, 9 aa, Artificial Sequence
  Neoantigenic peptide
TIPILTLSL

SEQ ID NO: 11 - protein, 9 aa, Artificial Sequence
  Neoantigenic peptide
GLRKTNMSL

SEQ ID NO: 12 - protein, 9 aa, Artificial Sequence
  Neoantigenic peptide
SMPANFETI

SEQ ID NO: 13 - protein, 9 aa, Artificial Sequence
  Neoantigenic peptide
STVRKSPWK

SEQ ID NO: 14 - protein, 9 aa, Artificial Sequence
  Neoantigenic peptide
STVRKSPWK

SEQ ID NO: 15 - protein, 9 aa, Artificial Sequence
  Neoantigen peptide
MGKSTHTSM

SEQ ID NO: 16 - protein, 9 aa, Artificial Sequence
  Neoantigen peptide
SMKAERPPA

SEQ ID NO: 17 - protein, 9 aa, Artificial Sequence
  Neoantigen peptide
TTSPSNTLV

SEQ ID NO: 18 - protein, 9 aa, Artificial Sequence
  Neoantigen peptide
SSSPTCSLM

SEQ ID NO: 19 - protein, 9 aa, Artificial Sequence
  Neoantigenic peptide
APLGAPPPL

SEQ ID NO: 20 - protein, 9 aa, Artificial Sequence
  neoantigenic peptide
ASLHHHHHR

SEQ ID NO: 21 - protein, 9 aa, Artificial Sequence
  neoantigenic peptide
ATYHFHFNL

SEQ ID NO: 22 - protein, 9 aa, Artificial Sequence
  neoantigenic peptide
DWPVFPGLF

SEQ ID NO: 23 - protein, 9 aa, Artificial Sequence
  neoantigenic peptide
EAFTLKATV

SEQ ID NO: 24 - protein, 9 aa, Artificial Sequence
  neoantigenic peptide
EAHHHFPSL

SEQ ID NO: 25 - protein, 9 aa, Artificial Sequence
  neoantigenic peptide
FLNRWMANT

SEQ ID NO: 26 - protein, 9 aa, Artificial Sequence
  neoantigenic peptide
GIVSWDTFL

SEQ ID NO: 27 - protein, 9 aa, Artificial Sequence
  neoantigenic peptide
GTPRAATMK

SEQ ID NO: 28 - protein, 9 aa, Artificial Sequence
  neoantigenic peptide
HWPEKEWPI

SEQ ID NO: 29 - protein, 9 aa, Artificial Sequence
  neoantigenic peptide
ILFDEAVKL

SEQ ID NO: 30 - protein, 9 aa, Artificial Sequence
  neoantigenic peptide
ILIACRLNK

SEQ ID NO: 31 - protein, 9 aa, Artificial Sequence
  neoantigenic peptide
ILPTCSPLV

SEQ ID NO: 32 - protein, 9 aa, Artificial Sequence
  neoantigenic peptide
KPRFLVGLW

SEQ ID NO: 33 - protein, 9 aa, Artificial Sequence
  neoantigenic peptide
KYIAFCINI

SEQ ID NO: 34 - protein, 9 aa, Artificial Sequence
  neoantigenic peptide
LFHQCLSIY

SEQ ID NO: 35 - protein, 9 aa, Artificial Sequence
  neoantigenic peptide
LLLMSTLGI

SEQ ID NO: 36 - protein, 9 aa, Artificial Sequence
  neoantigenic peptide
LLPPQDPHL

SEQ ID NO: 37 - protein, 9 aa, Artificial Sequence
  neoantigenic peptide
LQDFYLGTY

SEQ ID NO: 38 - protein, 9 aa, Artificial Sequence
  neoantigenic peptide
LTPPQAQEL

SEQ ID NO: 39 - protein, 9 aa, Artificial Sequence
  neoantigenic peptide
QTYQHMWNY

SEQ ID NO: 40 - protein, 9 aa, Artificial Sequence
  neoantigenic peptide
REFKFRVSA

SEQ ID NO: 41 - protein, 9 aa, Artificial Sequence
  neoantigenic peptide
STGFPHMLF

SEQ ID NO: 42 - protein, 9 aa, Artificial Sequence
  neoantigenic peptide
TLVGHQGPV

SEQ ID NO: 43 - protein, 9 aa, Artificial Sequence
  neoantigenic peptide
VDWFLDWLR

SEQ ID NO: 44 - protein, 9 aa, Artificial Sequence
  neoantigenic peptide
GGAPHFGHF

SEQ ID NO: 45 - protein, 9 aa, Artificial Sequence
  neoantigenic peptide
CYYELNQCL

SEQ ID NO: 46 - protein, 9 aa, Artificial Sequence
  neoantigenic peptide
AYPQYVIEY

SEQ ID NO: 47 - protein, 9 aa, Artificial Sequence
  neoantigenic peptide
HLETHNTDK

SEQ ID NO: 48 - protein, 9 aa, Artificial Sequence
  neoantigenic peptide
AEEEEEEVV

SEQ ID NO: 49 - protein, 9 aa, Artificial Sequence
  neoantigenic peptide
RGMQCAICK

SEQ ID NO: 50 - protein, 9 aa, Artificial Sequence
  neoantigenic peptide
MPEDEYMVY

SEQ ID NO: 51 - protein, 9 aa, Artificial Sequence
  neoantigenic peptide
SSYGRNHYI

SEQ ID NO: 52 - protein, 9 aa, Artificial Sequence
  neoantigenic peptide
AMDDLDTDM

SEQ ID NO: 53 - protein, 9 aa, Artificial Sequence
  neoantigenic peptide
PTDPMLGLA

SEQ ID NO: 54 - protein, 9 aa, Artificial Sequence
  neoantigenic peptide
FSSNLPTYY

SEQ ID NO: 55 - protein, 9 aa, Artificial Sequence
  neoantigenic peptide
FSSNLPTYY

SEQ ID NO: 56 - protein, 9 aa, Artificial Sequence
  neoantigenic peptide
FRHSMVVPY

SEQ ID NO: 57 - protein, 9 aa, Artificial Sequence
  neoantigenic peptide
NLLGRNSFK

SEQ ID NO: 58 - protein, 9 aa, Artificial Sequence
  neoantigenic peptide
GLGFYNDVV

SEQ ID NO: 59 - protein, 9 aa, Artificial Sequence
  neoantigenic peptide
AQTHEPRQW

SEQ ID NO: 60 - protein, 9 aa, Artificial Sequence
  neoantigenic peptide
STHPSLSQW

SEQ ID NO: 61 - protein, 9 aa, Artificial Sequence
  neoantigenic peptide
VYMPPPRLL

SEQ ID NO: 62 - protein, 9 aa, Artificial Sequence
  neoantigenic peptide
NHDDDDVEI

SEQ ID NO: 63 - protein, 9 aa, Artificial Sequence
  neoantigenic peptide
YVKIYLLPY

SEQ ID NO: 64 - protein, 9 aa, Artificial Sequence
  neoantigenic peptide
SYQSTGDPK

SEQ ID NO: 65 - protein, 9 aa, Artificial Sequence
  neoantigenic peptide
RPRKAWAWC

SEQ ID NO: 66 - protein, 9 aa, Artificial Sequence
  neoantigenic peptide
WVLHHMGGM

SEQ ID NO: 67 - protein, 9 aa, Artificial Sequence
  neoantigenic peptide
LAGEWRERL

SEQ ID NO: 68 - protein, 9 aa, Artificial Sequence
  neoantigenic peptide
TVWPSLAPL

SEQ ID NO: 69 - protein, 9 aa, Artificial Sequence
  neoantigenic peptide
QEASNKHAE

SEQ ID NO: 70 - protein, 9 aa, Artificial Sequence
  neoantigenic peptide
RRRLCILRM

SEQ ID NO: 71 - protein, 9 aa, Artificial Sequence
  neoantigenic peptide
VRLGPVKSI

SEQ ID NO: 72 - protein, 9 aa, Artificial Sequence
  neoantigenic peptide
FFVEKRHAF

SEQ ID NO: 73 - protein, 9 aa, Artificial Sequence
  neoantigenic peptide
HTSLRGFLY

SEQ ID NO: 74 - protein, 9 aa, Artificial Sequence
  neoantigenic peptide
SLAETKTLY

SEQ ID NO: 75 - protein, 9 aa, Artificial Sequence
  neoantigenic peptide
TYAPLFIWV

SEQ ID NO: 76 - protein, 9 aa, Artificial Sequence
  neoantigenic peptide
SPAPERCMV

SEQ ID NO: 77 - protein, 9 aa, Artificial Sequence
  neoantigenic peptide
EQLKLGAIF

SEQ ID NO: 78 - protein, 9 aa, Artificial Sequence
  neoantigenic peptide
RPQGQRPAL

SEQ ID NO: 79 - protein, 9 aa, Artificial Sequence
  neoantigenic peptide
APRGVCYGA

SEQ ID NO: 80 - protein, 9 aa, Artificial Sequence
  neoantigenic peptide
APRGVCYGA

SEQ ID NO: 81 - protein, 9 aa, Artificial Sequence
  neoantigenic peptide
LAAPRGVCY

SEQ ID NO: 82 - protein, 9 aa, Artificial Sequence
  neoantigenic peptide
PPRYIGIPI

SEQ ID NO: 83 - protein, 9 aa, Artificial Sequence
  neoantigenic peptide
HVWLCDLPV

SEQ ID NO: 84 - protein, 9 aa, Artificial Sequence
  neoantigenic peptide
QLYMNPKTW

SEQ ID NO: 85 - protein, 9 aa, Artificial Sequence
  neoantigenic peptide
KYSNYVWPI

SEQ ID NO: 86 - protein, 9 aa, Artificial Sequence
  neoantigenic peptide
LPRQYWEAL

SEQ ID NO: 87 - protein, 9 aa, Artificial Sequence
  neoantigenic peptide
VLNGWLRSV

SEQ ID NO: 88 - protein, 9 aa, Artificial Sequence
  neoantigenic peptide
YLALAAQCL

SEQ ID NO: 89 - protein, 9 aa, Artificial Sequence
  neoantigenic peptide
CPLPRPPPI

SEQ ID NO: 90 - protein, 9 aa, Artificial Sequence
  neoantigenic peptide
GIICLDYKL

SEQ ID NO: 91 - protein, 9 aa, Artificial Sequence
  neoantigenic peptide
TLGVFCLGL

SEQ ID NO: 92 - protein, 9 aa, Artificial Sequence
  neoantigenic peptide
ERPCHREPL

SEQ ID NO: 93 - protein, 9 aa, Artificial Sequence
  neoantigenic peptide
RLALSTFEW

SEQ ID NO: 94 - protein, 9 aa, Artificial Sequence
  neoantigenic peptide
VVWATKYFL

SEQ ID NO: 95 - protein, 9 aa, Artificial Sequence
  neoantigenic peptide
NPEAMCSDL

SEQ ID NO: 96 - protein, 9 aa, Artificial Sequence
  neoantigenic peptide
IPLEVMEPF

SEQ ID NO: 97 - protein, 9 aa, Artificial Sequence
  neoantigenic peptide
EEAFVPILY

SEQ ID NO: 98 - protein, 9 aa, Artificial Sequence
  neoantigenic peptide
HHHHHHQAW

SEQ ID NO: 99 - protein, 9 aa, Artificial Sequence
  neoantigenic peptide
LVWSLPCGF

SEQ ID NO: 100 - protein, 9 aa, Artificial Sequence
  neoantigenic peptide
MPDVVHQSL

SEQ ID NO: 101 - protein, 9 aa, Artificial Sequence
  neoantigenic peptide
CRPQCCQSV

SEQ ID NO: 102 - protein, 9 aa, Artificial Sequence
  neoantigenic peptide
MTPSVYGGA

SEQ ID NO: 103 - protein, 9 aa, Artificial Sequence
  neoantigenic peptide
YKLVVVGAV

SEQ ID NO: 104 - protein, 9 aa, Artificial Sequence
  neoantigenic peptide
YKLVVVGAV

SEQ ID NO: 105 - protein, 9 aa, Artificial Sequence
  neoantigenic peptide
YKLVVVGAV

SEQ ID NO: 106 - protein, 9 aa, Artificial Sequence
  neoantigenic peptide
APAQPPMLA

SEQ ID NO: 107 - protein, 9 aa, Artificial Sequence
  neoantigenic peptide
EPPPPPSPL

SEQ ID NO: 108 - protein, 9 aa, Artificial Sequence
  neoantigenic peptide
YLWEDPVCG

SEQ ID NO: 109 - protein, 9 aa, Artificial Sequence
  neoantigenic peptide
SFADFEWHF

SEQ ID NO: 110 - protein, 9 aa, Artificial Sequence
  neoantigenic peptide
YQQSNTWSL

SEQ ID NO: 111 - protein, 9 aa, Artificial Sequence
  neoantigenic peptide
SPGGWRSGW

SEQ ID NO: 112 - protein, 9 aa, Artificial Sequence
  neoantigenic peptide
RVWDIVPTL

SEQ ID NO: 113 - protein, 9 aa, Artificial Sequence
  neoantigenic peptide
MLAIGCALL

SEQ ID NO: 114 - protein, 9 aa, Artificial Sequence
  neoantigenic peptide
WEEEYTVWI

SEQ ID NO: 115 - protein, 9 aa, Artificial Sequence
  neoantigenic peptide
VWPKKINNI

SEQ ID NO: 116 - protein, 9 aa, Artificial Sequence
  neoantigenic peptide
WPQCHPEEI

SEQ ID NO: 117 - protein, 9 aa, Artificial Sequence
  neoantigenic peptide
QEFENIKSY

SEQ ID NO: 118 - protein, 9 aa, Artificial Sequence
  neoantigenic peptide
TMDVATPSV

SEQ ID NO: 119 - protein, 9 aa, Artificial Sequence
  neoantigenic peptide
LPLHLYDTL

SEQ ID NO: 120 - protein, 9 aa, Artificial Sequence
  neoantigenic peptide
RPGQSPGQL

SEQ ID NO: 121 - protein, 9 aa, Artificial Sequence
  neoantigenic peptide
ELLDYIRAV

SEQ ID NO: 122 - protein, 9 aa, Artificial Sequence
  neoantigenic peptide
LPPSLQGAV

SEQ ID NO: 123 - protein, 9 aa, Artificial Sequence
  neoantigenic peptide
FLTQPVAPK

SEQ ID NO: 124 - protein, 9 aa, Artificial Sequence
  neoantigenic peptide
LASSCGCTF

SEQ ID NO: 125 - protein, 9 aa, Artificial Sequence
  neoantigenic peptide
RPRGDNGYT

SEQ ID NO: 126 - protein, 9 aa, Artificial Sequence
  neoantigenic peptide
QAMYDVLTF

SEQ ID NO: 127 - protein, 9 aa, Artificial Sequence
  neoantigenic peptide
LTISGECPK

SEQ ID NO: 128 - protein, 9 aa, Artificial Sequence
  neoantigenic peptide
SWKSPGWSF

SEQ ID NO: 129 - protein, 9 aa, Artificial Sequence
  neoantigenic peptide
RKREEEERW

SEQ ID NO: 130 - protein, 9 aa, Artificial Sequence
  neoantigenic peptide
NHLCFGHCF

SEQ ID NO: 131 - protein, 9 aa, Artificial Sequence
  neoantigenic peptide
YVYSLYWSI

SEQ ID NO: 132 - protein, 9 aa, Artificial Sequence
  neoantigenic peptide
MVLWHLPAV

SEQ ID NO: 133 - protein, 9 aa, Artificial Sequence
  neoantigenic peptide
FSVSPEWAV

SEQ ID NO: 134 - protein, 9 aa, Artificial Sequence
  neoantigenic peptide
GYYTLLNVF

SEQ ID NO: 135 - protein, 9 aa, Artificial Sequence
  neoantigenic peptide
QALIRPTTF

SEQ ID NO: 136 - protein, 9 aa, Artificial Sequence
  neoantigenic peptide
KQLPRILEA

SEQ ID NO: 137 - protein, 9 aa, Artificial Sequence
  neoantigenic peptide
YQQALGKRF

SEQ ID NO: 138 - protein, 9 aa, Artificial Sequence
  neoantigenic peptide
QLAWVPSPY

SEQ ID NO: 139 - protein, 9 aa, Artificial Sequence
  neoantigenic peptide
HIQDLYTVL

SEQ ID NO: 140 - protein, 9 aa, Artificial Sequence
  neoantigenic peptide
MNRGRRSSL

SEQ ID NO: 141 - protein, 9 aa, Artificial Sequence
  neoantigenic peptide
YAYTFWTYI

SEQ ID NO: 142 - protein, 9 aa, Artificial Sequence
  neoantigenic peptide
SEVLGYWAF

SEQ ID NO: 143 - protein, 9 aa, Artificial Sequence
  neoantigenic peptide
KPLLSGPWA

SEQ ID NO: 144 - protein, 9 aa, Artificial Sequence
  neoantigenic peptide
FNGNFLLSM

SEQ ID NO: 145 - protein, 9 aa, Artificial Sequence
  neoantigenic peptide
AHPDGSWTF

SEQ ID NO: 146 - protein, 9 aa, Artificial Sequence
  neoantigenic peptide
MTTKATSSM

SEQ ID NO: 147 - protein, 9 aa, Artificial Sequence
  neoantigenic peptide
TLDYKPVTV

SEQ ID NO: 148 - protein, 9 aa, Artificial Sequence
  neoantigenic peptide
QIKNKNKEI

SEQ ID NO: 149 - protein, 9 aa, Artificial Sequence
  neoantigenic peptide
TLDYKPVTV

SEQ ID NO: 150 - protein, 9 aa, Artificial Sequence
  wild type epitope
PPSARGGPL

SEQ ID NO: 151 - protein, 9 aa, Artificial Sequence
  neoantigenic peptide
PPSARRGPL

SEQ ID NO: 152 - protein, 15 aa, Artificial Sequence
  Human Herpes Virus 8
PPSGQRGPVAFRTRV